European Patent Application EP 4 257 977 A1, published October 11, 2023. Title: An autoantibody associated with immunoglobulin A nephropathy. Applicant: JUNTENDO EDUCATIONAL FOUNDATION. The sequence listing filed with the application follows.

SEQUENCE LISTING (1 sequence)

SEQ ID NO: 13 - DNA, 13 bp, Artificial Sequence
aggtggaggcagc